European Patent Specification EP 4 045 533 B1, published November 15, 2023. Title: Human Monoclonal Antibodies to Severe Acute Respiratory Syndrome Corona Virus 2 (SARS-CoV-2). Applicant: Vanderbilt University Crowe, James E Jr. Zost, Seth Carnahan, Robert Gilchuk, Pavlo. The sequence listing filed with the application follows.

SEQUENCE LISTING (187 sequences)

SEQ ID NO: 1 - DNA, 351 bp, Artificial Sequence
  COV2-2165 Heavy
gaggtgcagctggtggagtctgggggaggcttggtccagcctggggggtctctgagactctcctgtgcagcctctggactcaccgtccgtagcaactacatgacctgggtccgccagactccagggaaggggctggaatgggtgtcagttatttatagcggtggtagcacattctacgcagactccgtgaagggcagattcaccatctccagagacaattccaagaacacggtgtatcttcaaatgaacagcctgagagccgaggacacggctgtgtattactgtgcgagagatctcgtgacttacggtttggacgtctggggccaagggaccacggtcaccgtctcctca

SEQ ID NO: 2 - DNA, 321 bp, Artificial Sequence
  COV2-2165 Light
gacatccagttgacccagtctccatccttcctgtctgcatctgtaggagacagagtcaccatcacttgccgggccagtcagggcattagcaattatttagcctggtatcagcaaaaaccagggacagcccctaacctcctgatctatgctgcatccactttgcaaagtggggtcccatcaaggttcagcggcagtggatctgggacagaattcactctcacaatcagcagcctgcagcctgaagattttgcaacttattactgtcaactacttaatagtcaccccctcaccttcggccaagggacacgactggagattaaa

SEQ ID NO: 3 - DNA, 370 bp, Artificial Sequence
  COV2-2838 Heavy
caaatgcagctggtgcagtctgggcctgaggtgaagaagcctgggacctcagtgaaggtctcctgcaaggcttctggattcacctttatgagctctgctgtgcagtgggtgcgacaggctcgtggacaacgccttgagtggataggatggatcgtcattggcagtggtaacacaaactacgcacagaagttccaggaaagagtcaccattaccagggacatgtccacaagcacagcctacatggagctgagcagcctgagatccgaggacacggccgtgtattactgtgcggccccatattgtagtagtatcagctgcaatgatggttttgatatctggggccaagggacaatggtcaccgtctcttcag

SEQ ID NO: 4 - DNA, 328 bp, Artificial Sequence
  COV2-2838 Light
gaaattgtgttgacgcagtctccaggcaccctgtctttgtctccaggggagagagccaccctctcctgcagggccagtcagagtgttagcagcagctacttagcctggtaccagcagaaacctggccaggctcccaggctcctcatctatggtgcatccagcagggccactggcatcccagacaggttcagtggcagtgggtctgggacagacttcactctcaccatcagcagactggagcctgaagattttgcagtgtattactgtcagcactatggtagctcacggggttggacgttcggccaagggaccaaggtggaaatcaaac

SEQ ID NO: 5 - DNA, 351 bp, Artificial Sequence; identical to SEQ ID NO: 1
  COV2-2952 heavy

SEQ ID NO: 6 - DNA, 322 bp, Artificial Sequence
  COV2-2952 light
gacatccagttgacccagtctccatccttcctgtctgcatctgtaggagacagagtcaccatcacttgccgggccagtcagggcattagcaattatttagcctggtatcagcaaaaaccagggacagcccctaacctcctgatctatgctgcatccactttgcaaagtggggtcccatcaaggttcagcggcagtggatctgggacagaattcactctcacaatcagcagcctgcagcctgaagattttgcaacttattactgtcaactacttaatagtcaccccctcaccttcggccaagggacacgactggagattaaac

SEQ ID NO: 7 - DNA, 388 bp, Artificial Sequence
  COV2-2514 heavy
gaggtgcagctggtggagtctgggggaggtgtggtacggcctggggggtccctgagactctcctgtgcagcctctggattcatctttgatgattatgacatgacctgggtccgccaagctccagggaaggggctggagtgggtctctggtattaattggaatggtggtagcacaggttatgcagactctgtgaagggccgattcaccatctccagagacaacgccaagaactccctgtatctgcaaatgaacagtctgagagccgaggacacggccttgtatcactgtgcagtgattatgtctccaatcccccgttatagtggctacgattgggcgggtgatgcttttgatatctggggccaagggacaatggtcaccgtctcttcag

SEQ ID NO: 8 - DNA, 325 bp, Artificial Sequence
  COV2-2514 light
tcttctgagctgactcaggaccctgctgtgtctgtggccttgggacagacagtcaggatcacatgccaaggagacagcctcagaagctattatgcaagttggtaccagcagaagccaggacaggtccctatacttgtcatctatgataaaaacaaccggccctcagggatcccagaccgattctctggctccagctcaggaaacacagcttccttgaccatcactggggctcaggcggaagatgaggctgactattactgtaactcccgggacagcagtggtaacgccgtggtattcggcggagggaccaagctgaccgtcctag

SEQ ID NO: 9 - DNA, 370 bp, Artificial Sequence
  COV2-2391 heavy
caggtgcagctggtgcagtctggggctgaggtgaagaagcctggggcctcagtgaaggtctcctgcaaggcttctggatacaccttcggcagctttgatatcaactgggtgcgacaggccactggacaagggcttgagtggatgggacggatgaactctaacagtgggaacacagcctatgcacagaagttccagggcagagtcactatgaccagggacacctccacaaatacagcctacatggagttgagcagcctgagatctgaggacacggccatgtattactgtgcgagaatgcgcagtggctggcccacacatggccgcccggatgacttctggggccggggaaccctggtcaccgtctcctcag

SEQ ID NO: 10 - DNA, 331 bp, Artificial Sequence
  COV2-2391 light
cagtctgtgctgactcaggcaccctcagcgtctgggacccccgggcagagggtcaccatctcttgttctggaagcaactccaatatcggaagttatactataaactggtaccagcagctcccaggaacggcccccaaactcctcatttatggtaatgatcagcggacctcaggggtccctgaccgattctctggctccaagtttggcacctcggcctccctggccatcagtgggctccagtctgaggatgaaaataattattactgtgcagtatgggatgacagcctgaatggcctggtattcggcggagggaccaaactgaccgtcctag

SEQ ID NO: 11 - DNA, 369 bp, Artificial Sequence
  COV2-3025 heavy
gaggtgcagctggtgcagtctgggcctgaggtgaagaagcctgggacctcagtgaaggtctcctgcaaggcttctggattcacctttatgagctctgctgtgcagtgggtgcgacaggctcgtggacaacgccttgagtggataggatggatcgtcattggcagtggtaacacaaactacgcacagaagttccaggaaagagtcaccattaccagggacatgtccacaagcacagcctacatggagctgagcagcctgagatccgaggacacggccgtgtattactgtgcggccccatattgtagtagtatcagctgcaatgatggttttgatatctggggccaagggacaatggtcaccgtctcttca

SEQ ID NO: 12 - DNA, 327 bp, Artificial Sequence
  COV2-3025 light
gaaattgtgttgacgcagtctccaggcaccctgtctttgtctccaggggagagagtcaccctctcctgcagggccagtcagagtgttagcagcagctacttagcctggtaccagcagaaacctggccaggctcccaggctcctcatctatggtgcatccagcagggccactggcatcccagacaggttcagtggcagtgggtctgggacagacttcactctcaccatcagcagactggagcctgaagattttgcagtgtattactgtcagcactatggtagctcacggggttggacgttcggccaagggaccaaggtggaaatcaaa

SEQ ID NO: 13 - DNA, 369 bp, Artificial Sequence
  COV2-2196 heavy
caaatgcagctggtgcagtctgggcctgaggtgaagaagcctgggacctcagtgaaggtctcctgcaaggcttctggattcacctttatgagctctgctgtgcagtgggtgcgacaggctcgtggacaacgccttgagtggataggatggatcgtcattggcagtggtaacacaaactacgcacagaagttccaggaaagagtcaccattaccagggacatgtccacaagcacagcctacatggagctgagcagcctgagatccgaggacacggccgtgtattactgtgcggccccatattgtagtagtatcagctgcaatgatggttttgatatctggggccaagggacaatggtcaccgtctcttca

SEQ ID NO: 14 - DNA, 327 bp, Artificial Sequence
  COV2-2196 light
gaaattgtgttgacgcagtctccaggcaccctgtctttgtctccaggggagagagccaccctctcctgcagggccagtcagagtgttagcagcagctacttagcctggtaccagcagaaacctggccaggctcccaggctcctcatctatggtgcatccagcagggccactggcatcccagacaggttcagtggcagtgggtctgggacagacttcactctcaccatcagcagactggagcctgaagattttgcagtgtattactgtcagcactatggtagctcacggggttggacgttcggccaagggaccaaggtggaaatcaaa

SEQ ID NO: 15 - DNA, 387 bp, Artificial Sequence
  COV2-2094 heavy
gaggtgcagctggtggagtctgggggaggtgtggtacggcctggggggtccctgagactctcctgtgcagcctctggattcatctttgatgattatgacatgacctgggtccgccaagctccagggaaggggctggagtgggtctctggtattaattggaatggtggtagcacaggttatgcagactctgtgaagggccgattcaccatctccagagacaacgccaagaactccctgtatctgcaaatgaacagtctgagagccgaggacacggccttgtatcactgtgcagtgattatgtctccaatcccccgttatagtggctacgattgggcgggtgatgcttttgatatctggggccaagggacaatggtcaccgtctcttca

SEQ ID NO: 16 - DNA, 324 bp, Artificial Sequence
  COV2-2094 light
tcttctgagctgactcaggaccctgctgtgtctgtggccttgggacagacagtcaggatcacatgccaaggagacagcctcagaagctattatgcaagttggtaccagcagaagccaggacaggtccctatacttgtcatctatgataaaaacaaccggccctcagggatcccagaccgattctctggctccagctcaggaaacacagcttccttgaccatcactggggctcaggcggaagatgaggctgactattactgtaactcccgggacagcagtggtaacgccgtggtattcggcggagggaccaagctgaccgtccta

SEQ ID NO: 17 - DNA, 369 bp, Artificial Sequence
  COV2-2096 heavy
caggtgcagctggtgcagtctggggctgaggtgaagaagcctggggcctcagtgaaggtctcctgcaaggcttctggatacaccttcggcagctttgatatcaactgggtgcgacaggccactggacaagggcttgagtggatgggacggatgaactctaacagtgggaacacagcctatgcacagaagttccagggcagagtcactatgaccagggacacctccacaaatacagcctacatggagttgagcagcctgagatctgaggacacggccatgtattactgtgcgagaatgcgcagtggctggcccacacatggccgcccggatgacttctggggccggggaaccctggtcaccgtctcctca

SEQ ID NO: 18 - DNA, 330 bp, Artificial Sequence
  COV2-2096 light
cagtctgtgctgactcaggcaccctcagcgtctgggacccccgggcagagggtcaccatctcttgttctggaagcaactccaatatcggaagttatactataaactggtaccagcagctcccaggaacggcccccaaactcctcatttatggtaatgatcagcggacctcaggggtccctgaccgattctctggctccaagtttggcacctcggcctccctggccatcagtgggctccagtctgaggatgaaaataattattactgtgcagtatgggatgacagcctgaatggcctggtattcggcggagggaccaaactgaccgtccta

SEQ ID NO: 19 - DNA, 393 bp, Artificial Sequence
  COV2-2130 heavy
gaggtgcagctggtggagtctgggggaggcttggtaaagcctggggggtcccttagactctcctgtgcagcctctggattcactttcagagacgtctggatgagctgggtccgccaggctccagggaaggggctggagtgggttggccgtattaaaagcaaaattgatggtgggacaacagactacgctgcacccgtgaaaggcagattcaccatctcaagagatgattcaaaaaacacgctgtatctgcaaatgaacagcctgaaaaccgaggacacagccgtgtattactgtaccacagcgggaagctattactatgatactgttggtccaggcctcccagagggaaaatttgactactggggccagggaaccctggtcaccgtctcctca

SEQ ID NO: 20 - DNA, 336 bp, Artificial Sequence
  COV2-2130 light
gacatcgtgatgacccagtctccagactccctggctgtgtctctgggcgagagggccaccatcaactgcaagtccagccagagtgttttatacagctccaacaataagaactacttagcttggtaccagcagaaaccaggacagcctcctaagctgctcatgtactgggcatctacccgggaatccggggtccctgaccgattcagtggcagcgggtctggggcagagttcactctcaccatcagcagcctgcaggctgaagatgtggcaatttattactgtcagcaatattatagtaccctcactttcggcggagggaccaaggtggagatcaaa

SEQ ID NO: 21 - protein, 117 aa, Artificial Sequence
  COV2-2165 heavy
EVQLVESGGGLVQPGGSLRLSCAASGLTVRSNYMTWVRQTPGKGLEWVSVIYSGGSTFYADSVKGRFTISRDNSKNTVYLQMNSLRAEDTAVYYCARDLVTYGLDVWGQGTTVTVSS

SEQ ID NO: 22 - protein, 107 aa, Artificial Sequence
  COV2-2165 light
DIQLTQSPSFLSASVGDRVTITCRASQGISNYLAWYQQKPGTAPNLLIYAASTLQSGVPSRFSGSGSGTEFTLTISSLQPEDFATYYCQLLNSHPLTFGQGTRLEIK

SEQ ID NO: 23 - protein, 123 aa, Artificial Sequence
  COV2-2838 heavy
QMQLVQSGPEVKKPGTSVKVSCKASGFTFMSSAVQWVRQARGQRLEWIGWIVIGSGNTNYAQKFQERVTITRDMSTSTAYMELSSLRSEDTAVYYCAAPYCSSISCNDGFDIWGQGTMVTVSS

SEQ ID NO: 24 - protein, 109 aa, Artificial Sequence
  COV2-2838 light
EIVLTQSPGTLSLSPGERATLSCRASQSVSSSYLAWYQQKPGQAPRLLIYGASSRATGIPDRFSGSGSGTDFTLTISRLEPEDFAVYYCQHYGSSRGWTFGQGTKVEIK

SEQ ID NO: 25 - protein, 117 aa, Artificial Sequence; identical to SEQ ID NO: 21
  COV2-2952 heavy

SEQ ID NO: 26 - protein, 107 aa, Artificial Sequence; identical to SEQ ID NO: 22
  COV2-2952 light

SEQ ID NO: 27 - protein, 129 aa, Artificial Sequence
  COV2-2514 heavy
EVQLVESGGGVVRPGGSLRLSCAASGFIFDDYDMTWVRQAPGKGLEWVSGINWNGGSTGYADSVKGRFTISRDNAKNSLYLQMNSLRAEDTALYHCAVIMSPIPRYSGYDWAGDAFDIWGQGTMVTVSS

SEQ ID NO: 28 - protein, 108 aa, Artificial Sequence
  COV2-2514 light
SSELTQDPAVSVALGQTVRITCQGDSLRSYYASWYQQKPGQVPILVIYDKNNRPSGIPDRFSGSSSGNTASLTITGAQAEDEADYYCNSRDSSGNAVVFGGGTKLTVL

SEQ ID NO: 29 - protein, 123 aa, Artificial Sequence
  COV2-2391 heavy
QVQLVQSGAEVKKPGASVKVSCKASGYTFGSFDINWVRQATGQGLEWMGRMNSNSGNTAYAQKFQGRVTMTRDTSTNTAYMELSSLRSEDTAMYYCARMRSGWPTHGRPDDFWGRGTLVTVSS

SEQ ID NO: 30 - protein, 110 aa, Artificial Sequence
  COV2-2391 light
QSVLTQAPSASGTPGQRVTISCSGSNSNIGSYTINWYQQLPGTAPKLLIYGNDQRTSGVPDRFSGSKFGTSASLAISGLQSEDENNYYCAVWDDSLNGLVFGGGTKLTVL

SEQ ID NO: 31 - protein, 123 aa, Artificial Sequence
  COV2-3025 heavy
EVQLVQSGPEVKKPGTSVKVSCKASGFTFMSSAVQWVRQARGQRLEWIGWIVIGSGNTNYAQKFQERVTITRDMSTSTAYMELSSLRSEDTAVYYCAAPYCSSISCNDGFDIWGQGTMVTVSS

SEQ ID NO: 32 - protein, 109 aa, Artificial Sequence
  COV2-3025 light
EIVLTQSPGTLSLSPGERVTLSCRASQSVSSSYLAWYQQKPGQAPRLLIYGASSRATGIPDRFSGSGSGTDFTLTISRLEPEDFAVYYCQHYGSSRGWTFGQGTKVEIK

SEQ ID NO: 33 - protein, 123 aa, Artificial Sequence; identical to SEQ ID NO: 23
  COV2-2196 heavy

SEQ ID NO: 34 - protein, 109 aa, Artificial Sequence; identical to SEQ ID NO: 24
  COV2-2196 light

SEQ ID NO: 35 - protein, 129 aa, Artificial Sequence; identical to SEQ ID NO: 27
  COV2-2094 heavy

SEQ ID NO: 36 - protein, 108 aa, Artificial Sequence; identical to SEQ ID NO: 28
  COV2-2094 light

SEQ ID NO: 37 - protein, 123 aa, Artificial Sequence; identical to SEQ ID NO: 29
  COV2-2096 heavy

SEQ ID NO: 38 - protein, 110 aa, Artificial Sequence; identical to SEQ ID NO: 30
  COV2-2096 light

SEQ ID NO: 39 - protein, 131 aa, Artificial Sequence
  COV2-2130 heavy
EVQLVESGGGLVKPGGSLRLSCAASGFTFRDVWMSWVRQAPGKGLEWVGRIKSKIDGGTTDYAAPVKGRFTISRDDSKNTLYLQMNSLKTEDTAVYYCTTAGSYYYDTVGPGLPEGKFDYWGQGTLVTVSS

SEQ ID NO: 40 - protein, 112 aa, Artificial Sequence
  COV2-2130 light
DIVMTQSPDSLAVSLGERATINCKSSQSVLYSSNNKNYLAWYQQKPGQPPKLLMYWASTRESGVPDRFSGSGSGAEFTLTISSLQAEDVAIYYCQQYYSTLTFGGGTKVEIK

SEQ ID NO: 41 - protein, 8 aa, Artificial Sequence
  COV2-2165 CDRH1
GLTVRSNY

SEQ ID NO: 42 - protein, 7 aa, Artificial Sequence
  COV2-2165 CDRH2
IYSGGST

SEQ ID NO: 43 - protein, 11 aa, Artificial Sequence
  COV2-2165 CDRH3
ARDLVTYGLDV

SEQ ID NO: 44 - protein, 8 aa, Artificial Sequence
  COV2-2838 CDRH1
GFTFMSSA

SEQ ID NO: 45 - protein, 8 aa, Artificial Sequence
  COV2-2838 CDRH2
IVIGSGNT

SEQ ID NO: 46 - protein, 16 aa, Artificial Sequence
  COV2-2838 CDRH3
AAPYCSSISCNDGFDI

SEQ ID NO: 47 - protein, 8 aa, Artificial Sequence
  COV2-2952 CDRH1
GLTVRSNY

SEQ ID NO: 48 - protein, 7 aa, Artificial Sequence
  COV2-2952 CDRH2
IYSGGST

SEQ ID NO: 49 - protein, 11 aa, Artificial Sequence
  COV2-2952 CDRH3
ARDLVTYGLDV

SEQ ID NO: 50 - protein, 8 aa, Artificial Sequence
  COV2-2514 CDRH1
GFIFDDYD

SEQ ID NO: 51 - protein, 8 aa, Artificial Sequence
  COV2-2514 CDRH2
INWNGGST

SEQ ID NO: 52 - protein, 22 aa, Artificial Sequence
  COV2-2514 CDRH3
AVIMSPIPRYSGYDWAGDAFDI

SEQ ID NO: 53 - protein, 8 aa, Artificial Sequence
  COV2-2391 CDRH1
GYTFGSFD

SEQ ID NO: 54 - protein, 8 aa, Artificial Sequence
  COV2-2391 CDRH2
MNSNSGNT

SEQ ID NO: 55 - protein, 16 aa, Artificial Sequence
  COV2-2391 CDRH3
ARMRSGWPTHGRPDDF

SEQ ID NO: 56 - protein, 8 aa, Artificial Sequence
  COV2-3025 CDRH1
GFTFMSSA

SEQ ID NO: 57 - protein, 8 aa, Artificial Sequence
  COV2-3025 CDRH2
IVIGSGNT

SEQ ID NO: 58 - protein, 16 aa, Artificial Sequence
  COV2-3025 CDRH3
AAPYCSSISCNDGFDI

SEQ ID NO: 59 - protein, 8 aa, Artificial Sequence
  COV2-2196 CDRH1
GFTFMSSA

SEQ ID NO: 60 - protein, 8 aa, Artificial Sequence
  COV2-2196 CDRH2
IVIGSGNT

SEQ ID NO: 61 - protein, 16 aa, Artificial Sequence
  COV2-2196 CDRH3
AAPYCSSISCNDGFDI

SEQ ID NO: 62 - protein, 8 aa, Artificial Sequence
  COV2-2094 CDRH1
GFIFDDYD

SEQ ID NO: 63 - protein, 8 aa, Artificial Sequence
  COV2-2094 CDRH2
INWNGGST

SEQ ID NO: 64 - protein, 22 aa, Artificial Sequence
  COV2-2094 CDRH3
AVIMSPIPRYSGYDWAGDAFDI

SEQ ID NO: 65 - protein, 8 aa, Artificial Sequence
  COV2-2096 CDRH1
GYTFGSFD

SEQ ID NO: 66 - protein, 8 aa, Artificial Sequence
  COV2-2096 CDRH2
MNSNSGNT

SEQ ID NO: 67 - protein, 16 aa, Artificial Sequence
  COV2-2096 CDRH3
ARMRSGWPTHGRPDDF

SEQ ID NO: 68 - protein, 8 aa, Artificial Sequence
  COV2-2130 CDRH1
GFTFRDVW

SEQ ID NO: 69 - protein, 10 aa, Artificial Sequence
  COV2-2130 CDRH2
IKSKIDGGTT

SEQ ID NO: 70 - protein, 22 aa, Artificial Sequence
  COV2-2130 CDRH3
TTAGSYYYDTVGPGLPEGKFDY

SEQ ID NO: 71 - protein, 6 aa, Artificial Sequence
  COV2-2165 CDRL1
QGISNY

SEQ ID NO: 72 - protein, 3 aa, Artificial Sequence
  COV2-2165 CDRL2
AAS

SEQ ID NO: 73 - protein, 9 aa, Artificial Sequence
  COV2-2165 CDRL3
QLLNSHPLT

SEQ ID NO: 74 - protein, 7 aa, Artificial Sequence
  COV2-2838 CDRL1
QSVSSSY

SEQ ID NO: 75 - protein, 3 aa, Artificial Sequence
  COV2-2838 CDRL2
GAS

SEQ ID NO: 76 - protein, 10 aa, Artificial Sequence
  COV2-2838 CDRL3
QHYGSSRGWT

SEQ ID NO: 77 - protein, 6 aa, Artificial Sequence
  COV2-2952 CDRL1
QGISNY

SEQ ID NO: 78 - protein, 3 aa, Artificial Sequence
  COV2-2952 CDRL2
AAS

SEQ ID NO: 79 - protein, 9 aa, Artificial Sequence
  COV2-2952 CDRL3
QLLNSHPLT

SEQ ID NO: 80 - protein, 6 aa, Artificial Sequence
  COV2-2514 CDRL1
SLRSYY

SEQ ID NO: 81 - protein, 3 aa, Artificial Sequence
  COV2-2514 CDRL2
DKN

SEQ ID NO: 82 - protein, 11 aa, Artificial Sequence
  COV2-2514 CDRL3
NSRDSSGNAVV

SEQ ID NO: 83 - protein, 8 aa, Artificial Sequence
  COV2-2391 CDRL1
NSNIGSYT

SEQ ID NO: 84 - protein, 3 aa, Artificial Sequence
  COV2-2391 CDRL2
GND

SEQ ID NO: 85 - protein, 11 aa, Artificial Sequence
  COV2-2391 CDRL3
AVWDDSLNGLV

SEQ ID NO: 86 - protein, 7 aa, Artificial Sequence
  COV2-3025 CDRL1
QSVSSSY

SEQ ID NO: 87 - protein, 3 aa, Artificial Sequence
  COV2-3025 CDRL2
GAS

SEQ ID NO: 88 - protein, 10 aa, Artificial Sequence
  COV2-3025 CDRL3
QHYGSSRGWT

SEQ ID NO: 89 - protein, 7 aa, Artificial Sequence
  COV2-2196 CDRL1
QSVSSSY

SEQ ID NO: 90 - protein, 3 aa, Artificial Sequence
  COV2-2196 CDRL2
GAS

SEQ ID NO: 91 - protein, 10 aa, Artificial Sequence
  COV2-2196 CDRL3
QHYGSSRGWT

SEQ ID NO: 92 - protein, 6 aa, Artificial Sequence
  COV2-2094 CDRL1
SLRSYY

SEQ ID NO: 93 - protein, 3 aa, Artificial Sequence
  COV2-2094 CDRL2
DKN

SEQ ID NO: 94 - protein, 11 aa, Artificial Sequence
  COV2-2094 CDRL3
NSRDSSGNAVV

SEQ ID NO: 95 - protein, 8 aa, Artificial Sequence
  COV2-2096 CDRL1
NSNIGSYT

SEQ ID NO: 96 - protein, 3 aa, Artificial Sequence
  COV2-2096 CDRL2
GND

SEQ ID NO: 97 - protein, 11 aa, Artificial Sequence
  COV2-2096 CDRL3
AVWDDSLNGLV

SEQ ID NO: 98 - protein, 12 aa, Artificial Sequence
  COV2-2130 CDRL1
QSVLYSSNNKNY

SEQ ID NO: 99 - protein, 3 aa, Artificial Sequence
  COV2-2130 CDRL2
WAS

SEQ ID NO: 100 - protein, 8 aa, Artificial Sequence
  COV2-2130 CDRL3
QQYYSTLT

SEQ ID NO: 101 - protein, 5 aa, Artificial Sequence
  IGHV1-58 FR2-HCDR2
IGWIV

SEQ ID NO: 102 - protein, 3 aa, Artificial Sequence
  IGHV1-58 HCDR3-FR4
CAA

SEQ ID NO: 103 - protein, 10 aa, Artificial Sequence
  IGHD2-2 HCDR3-FR4
GYCSSTSCYA

SEQ ID NO: 104 - protein, 10 aa, Artificial Sequence
  IGHD2-8 HCDR3-FR4
GYCTNGVCYA

SEQ ID NO: 105 - protein, 10 aa, Artificial Sequence
  IGHD2-15 HCDR3-FR4
GYCSGGSCYS

SEQ ID NO: 106 - protein, 6 aa, Artificial Sequence
  IGHJ3*02 HCDR3-FR4
DAFDIW

SEQ ID NO: 107 - protein, 6 aa, Artificial Sequence
  IGKV3-20 LCDR1-FR2
SSYLAW

SEQ ID NO: 108 - protein, 6 aa, Artificial Sequence
  IGKV3-20 LCDR3-FR4
QYGSSP

SEQ ID NO: 109 - protein, 4 aa, Artificial Sequence
  IGKJ1*01 LCDR3-FR4
WTFG

SEQ ID NO: 110 - protein, 5 aa, Artificial Sequence
  COV2-2196 FR2-HCDR2
IGWIV

SEQ ID NO: 111 - protein, 18 aa, Artificial Sequence
  COV2-2196 HCDR3-FR4
CAAPYCSSISCNDGFDIW

SEQ ID NO: 112 - protein, 6 aa, Artificial Sequence
  COV2-2196 LCDR1-FR2
SSYLAW

SEQ ID NO: 113 - protein, 11 aa, Artificial Sequence
  COV2-2196 LCDR3-FR4
HYGSSRGWTFG

SEQ ID NO: 114 - protein, 5 aa, Artificial Sequence
  COV2-2381 FR2-HCDR2
IGWIA

SEQ ID NO: 115 - protein, 18 aa, Artificial Sequence
  COV2-2381 HCDR3-FR4
CAAPYCSRTSCHDAFDIW

SEQ ID NO: 116 - protein, 6 aa, Artificial Sequence
  COV2-2381 LCDR1-FR2
SSYLAW

SEQ ID NO: 117 - protein, 11 aa, Artificial Sequence
  COV2-2381 LCDR3-FR4
HFGSSSQWTFG

SEQ ID NO: 118 - protein, 5 aa, Artificial Sequence
  COV2-2072 FR2-HCDR2
IGWIV

SEQ ID NO: 119 - protein, 18 aa, Artificial Sequence
  COV2-2072 HCDR3-FR4
CAAPHCNRTSCYDAFDLW

SEQ ID NO: 120 - protein, 6 aa, Artificial Sequence
  COV2-2072 LCDR1-FR2
SSYLGW

SEQ ID NO: 121 - protein, 10 aa, Artificial Sequence
  COV2-2072 LCDR3-FR4
QYGSSPWTFG

SEQ ID NO: 122 - protein, 5 aa, Artificial Sequence
  MnC5t2p1_G1 FR2-HCDR2
IGWIV

SEQ ID NO: 123 - protein, 18 aa, Artificial Sequence
  MnC5t2p1_G1 HCDR3-FR4
CAAPRCSGGSCYDGFDIW

SEQ ID NO: 124 - protein, 6 aa, Artificial Sequence
  MnC5t2p1_G1 LCDR1-FR2
SSYLAW

SEQ ID NO: 125 - protein, 10 aa, Artificial Sequence
  MnC5t2p1_G1 LCDR3-FR4
QYGSSPWTFG

SEQ ID NO: 126 - protein, 5 aa, Artificial Sequence
  HbnC3t1p2_C6 FR2-HCDR2
IGWIV

SEQ ID NO: 127 - protein, 18 aa, Artificial Sequence
  HbnC3t1p2_C6 HCDR3-FR4
CAAPYCSSTRCYDAFDIW

SEQ ID NO: 128 - protein, 6 aa, Artificial Sequence
  HbnC3t1p2_C6 LCDR1-FR2
SSYLAW

SEQ ID NO: 129 - protein, 10 aa, Artificial Sequence
  HbnC3t1p2_C6 LCDR3-FR4
QYGRSPWTFG

SEQ ID NO: 130 - protein, 5 aa, Artificial Sequence
  HbnC3t1p1_C6 FR2-HCDR2
IGWIV

SEQ ID NO: 131 - protein, 18 aa, Artificial Sequence
  HbnC3t1p1_C6 HCDR3-FR4
CAAPHCSSTICYDGFDIW

SEQ ID NO: 132 - protein, 6 aa, Artificial Sequence
  HbnC3t1p1_C6 LCDR1-FR2
SSYLAW

SEQ ID NO: 133 - protein, 10 aa, Artificial Sequence
  HbnC3t1p1_C6 LCDR3-FR4
QYGSSPWTFG

SEQ ID NO: 134 - protein, 5 aa, Artificial Sequence
  S2E12 FR2-HCDR2
VGWIV

SEQ ID NO: 135 - protein, 18 aa, Artificial Sequence
  S2E12 HCDR3-FR4
CASPYCSGGSCSDGFDIW

SEQ ID NO: 136 - protein, 6 aa, Artificial Sequence
  S2E12 LCDR1-FR2
SSYLAW

SEQ ID NO: 137 - protein, 11 aa, Artificial Sequence
  S2E12 LCDR3-FR4
QYVGLTGWTFG

SEQ ID NO: 138 - protein, 5 aa, Artificial Sequence
  COV107_1 FR2-HCDR2
IGWIV

SEQ ID NO: 139 - protein, 18 aa, Artificial Sequence
  COV107_1 HCDR3-FR4
CAAPHCSSTSCFDAFDIW

SEQ ID NO: 140 - protein, 6 aa, Artificial Sequence
  COV107_1 LCDR1-FR2
SSYLAW

SEQ ID NO: 141 - protein, 10 aa, Artificial Sequence
  COV107_1 LCDR3-FR4
QYGNSPWTFG

SEQ ID NO: 142 - protein, 5 aa, Artificial Sequence
  COV107_2 FR2-HCDR2
IGWIV

SEQ ID NO: 143 - protein, 18 aa, Artificial Sequence
  COV107_2 HCDR3-FR4
CAAPYCSGGSCSDAFDIW

SEQ ID NO: 144 - protein, 6 aa, Artificial Sequence
  COV107_2 LCDR1-FR2
SSYLAW

SEQ ID NO: 145 - protein, 10 aa, Artificial Sequence
  COV107_2 LCDR3-FR4
QYGSSPWTFG

SEQ ID NO: 146 - protein, 5 aa, Artificial Sequence
  COV72 FR2-HCDR2
IGWIV

SEQ ID NO: 147 - protein, 18 aa, Artificial Sequence
  COV72 HCDR3-FR4
CAAVDCNSTSCYDAFDIW

SEQ ID NO: 148 - protein, 6 aa, Artificial Sequence
  COV72 LCDR1-FR2
SSYLAW

SEQ ID NO: 149 - protein, 10 aa, Artificial Sequence
  COV72 LCDR3-FR4
QYDISPWTFG

SEQ ID NO: 150 - protein, 5 aa, Artificial Sequence
  COV21_1 FR2-HCDR2
IGWIV

SEQ ID NO: 151 - protein, 18 aa, Artificial Sequence
  COV21_1 HCDR3-FR4
CAAPHCSGGSCLDAFDIW

SEQ ID NO: 152 - protein, 6 aa, Artificial Sequence
  COV21_1 LCDR1-FR2
SSYLAW

SEQ ID NO: 153 - protein, 10 aa, Artificial Sequence
  COV21_1 LCDR3-FR4
QYGSSPWTFG

SEQ ID NO: 154 - protein, 5 aa, Artificial Sequence
  COV21_2 FR2-HCDR2
IGWIV

SEQ ID NO: 155 - protein, 18 aa, Artificial Sequence
  COV21_2 HCDR3-FR4
CAAPHCSGGSCYDAFDIW

SEQ ID NO: 156 - protein, 6 aa, Artificial Sequence
  COV21_2 LCDR1-FR2
SSYLAW

SEQ ID NO: 157 - protein, 10 aa, Artificial Sequence
  COV21_2 LCDR3-FR4
QYGSSPWTFG

SEQ ID NO: 158 - protein, 5 aa, Artificial Sequence
  COV57_1 FR2-HCDR2
IGWIV

SEQ ID NO: 159 - protein, 18 aa, Artificial Sequence
  COV57_1 HCDR3-FR4
CAANHCSGGSCYDGFDIW

SEQ ID NO: 160 - protein, 6 aa, Artificial Sequence
  COV57_1 LCDR1-FR2
SSYLAW

SEQ ID NO: 161 - protein, 10 aa, Artificial Sequence
  COV57_1 LCDR3-FR4
QYGSSPWMFG

SEQ ID NO: 162 - protein, 5 aa, Artificial Sequence
  COV57_2 FR2-HCDR2
IGWIV

SEQ ID NO: 163 - protein, 18 aa, Artificial Sequence
  COV57_2 HCDR3-FR4
CAAPYCSGGSCNDAFDIW

SEQ ID NO: 164 - protein, 6 aa, Artificial Sequence
  COV57_2 LCDR1-FR2
SSYLAW

SEQ ID NO: 165 - protein, 10 aa, Artificial Sequence
  COV57_2 LCDR3-FR4
QYGSSPWTFG

SEQ ID NO: 166 - protein, 129 aa, Artificial Sequence
  HIP1 HEAVY CHAIN
  MISC_FEATURE (81)..(81): Xaa can be Met, Val
  MISC_FEATURE (100)..(100): Xaa can be Trp, Ser, Arg
  MISC_FEATURE (101)..(101): Xaa can be Asp, Arg, Val
  MISC_FEATURE (102)..(102): Xaa can be Leu, Arg, Ala
  MISC_FEATURE (103)..(103): Xaa can be Ala, Gly
  MISC_FEATURE (104)..(104): Xaa can be Tyr, Ile
  MISC_FEATURE (107)..(107): Xaa can be Val, Cys
  MISC_FEATURE (108)..(108): Xaa can be Val, Tyr, Thr
  MISC_FEATURE (109)..(109): Xaa can be Gly, Val
  MISC_FEATURE (110)..(110): Xaa can be Asp, Val
  MISC_FEATURE (111)..(111): Xaa can be Cys, Ala
  MISC_FEATURE (112)..(112): Xaa can be Ser, Thr
  MISC_FEATURE (113)..(113): Xaa can be Arg, His, Ala
QMQLVQSGPEVKKPGTSVKVSCKASGFTFTSSAVQWVRQARGQRLEWIGWIVVGSGNTNYAQKFQERVTITRDMSTSTAYXELSSLRSEDTAVYYCAAPXXXXXCGXXXXXXXDAFDIWGQGTMVTVSS

SEQ ID NO: 167 - protein, 128 aa, Artificial Sequence
  HIP2 HEAVY CHAIN
  misc_feature (3)..(3): Xaa can be Gln, Pro
  misc_feature (4)..(4): Xaa can be Leu, Arg
  misc_feature (34)..(34): Xaa can be Met, Val
  misc_feature (100)..(100): Xaa can be Gly, Asn, Asp, Gln, Thr, Ser, Leu, Arg
  misc_feature (101)..(101): Xaa can be Pro, Gly, Leu, Ser, Val, Lys, Ala
  misc_feature (102)..(102): Xaa can be Ser, Gly, Ile, Val, Arg, Pro, Ala, Met
  misc_feature (103)..(103): Xaa can be Tyr, Leu, Ile, Arg, Asn, Ala
  misc_feature (104)..(104): Xaa can be Cys, Ser, Val, Tyr
  misc_feature (105)..(105): Xaa can be Ser, Arg, Val, Tyr, Met
  misc_feature (106)..(106): Xaa can be Ser, Gly, Val, Cys
  misc_feature (107)..(107): Xaa can be Gly, Thr
  misc_feature (108)..(108): Xaa can be Ser, Gly, Val, Thr
  misc_feature (109)..(109): Xaa can be Cys, Ala, Thr, Asp
  misc_feature (110)..(110): Xaa can be Tyr, Arg, Phe, Pro, Thr
  misc_feature (111)..(111): Xaa can be Ala, Pro, Gly, Val, Cys, Arg
  misc_feature (112)..(112): Xaa can be Asp, Thr, Ser, Asn, Leu, Ile, Tyr, Pro
QMXXVQSGPEVKKPGTSVKVSCKASGFTFTSSAXQWVRQARGQRLEWIGWIVVGSGNTNYAQKFQERVTITRDMSTSTAYMELSSLRSEDTAVYYCAAPXXXXXXXXXXXXXDAFDIWGQGTMVTVSS

SEQ ID NO: 168 - protein, 129 aa, Artificial Sequence
  HIP3 HEAVY CHAIN
  misc_feature (3)..(3): Xaa can be Gln, Pro
  misc_feature (34)..(34): Xaa can be Met or Val
  misc_feature (35)..(35): Xaa can be Gln, Arg
  misc_feature (43)..(43): Xaa can be Gln, Arg
  misc_feature (100)..(100): Xaa can be Tyr, Pro, Ala, Arg, Gly
  misc_feature (101)..(101): Xaa can be Glu, Leu, Pro, Tyr, Ser
  misc_feature (102)..(102): Xaa can be Gly, Val, Ser, Cys, Tyr
  misc_feature (103)..(103): Xaa can be Cys, Asp, Val, Gln, Thr
  misc_feature (104)..(104): Xaa can be Gly, Asn
  misc_feature (106)..(106): Xaa can be Asp, Val
  misc_feature (108)..(108): Xaa can be Tyr, Ala, His
  misc_feature (109)..(109): Xaa can be Thr, Gln, Ser
  misc_feature (110)..(110): Xaa can be Val, His
  misc_feature (111)..(111): Xaa can be Thr, Arg
  misc_feature (112)..(112): Xaa can be Ala, Pro
  misc_feature (113)..(113): Xaa can be Leu, Phe, Ala, Gly, Asn
QMXLVQSGPEVKKPGTSVKVSCKASGFTFTSSAXXWVRQARGXRLEWIGWIVVGSGNTNYAQKFQERVTITRDMSTSTAYMELSSLRSEDTAVYYCAAPXXXXXGXCXXXXXXDAFDIWGQGTMVTVSS

SEQ ID NO: 169 - protein, 106 aa, Artificial Sequence
  CORD HEAVY CHAIN
  misc_feature (19)..(19): Xaa can be Arg, Leu
  misc_feature (78)..(78): Xaa can be Val, Glu, Gly
  misc_feature (79)..(79): Xaa can be Pro, Gly, or His
  misc_feature (80)..(80): Xaa can be Cys, Ile, Tyr
  misc_feature (81)..(81): Xaa can be Ser, Cys, Val
  misc_feature (85)..(85): Xaa can be Cys, Ser, Val
  misc_feature (86)..(86): Xaa can be Tyr, Ser, Val
  misc_feature (87)..(87): Xaa can be Ser, Thr, Val
  misc_feature (88)..(88): Xaa can be Tyr, Ala, Ser
  misc_feature (89)..(89): Xaa can be Ser, Ala, Cys
  misc_feature (90)..(90): Xaa can be Asp, Tyr
KASGFTFTSSAVQWVRQAXGQRLEWIGWIVVGSGNTNYAQKFQERVTITRDMSTSTAYMELSSLRSEDTAVYYCAAPXXXXGGSXXXXXXDAFDIWGQGTMVTVSS

SEQ ID NO: 170 - protein, 109 aa, Artificial Sequence
  HIP1 LIGHT CHAIN
  misc_feature (97)..(97): Xaa can be Pro, Leu, Ser, Thr
EIVLTQSPGTLSLSPGERATLSCRASQSVSSSYLAWYQQKPGQAPRLLIYGASSRATGIPDRFSGSGSGTDFTLTISRLEPEDFAVYYCQQYGSSPXWTFGQGTKVEIK

SEQ ID NO: 171 - protein, 109 aa, Artificial Sequence; identical to SEQ ID NO: 170
  HIP2 LIGHT CHAIN
  misc_feature (97)..(97): Xaa can be Pro, Leu, Ser, Thr

SEQ ID NO: 172 - protein, 109 aa, Artificial Sequence; identical to SEQ ID NO: 170
  HIP3 LIGHT CHAIN
  misc_feature (97)..(97): Xaa can be Pro, Leu, Ser, Thr

SEQ ID NO: 173 - protein, 108 aa, Artificial Sequence
  HIP1 Light Chain
EIVLTQSPGTLSLSPGERATLSCRASQSVSSSYLAWYQQKPGQAPRLLIYGASSRATGIPDRFSGSGSGTDFTLTISRLEPEDFAVYYCQQYGSSPWTFGQGTKVEIK

SEQ ID NO: 174 - protein, 109 aa, Artificial Sequence
  HIP1 Light Chain
EIVLTQSPGTLSLSPGERATLSCRASQSVSSSYLAWYQQKPGQAPRLLIYGASSRATGIPDRFSGSGSGTDFTLTISRLEPEDFAVYYCQQYGSSPPWTFGQGTKVEIK

SEQ ID NO: 175 - protein, 108 aa, Artificial Sequence
  HIP1 Light Chain
EIVLTQSPGTLSLSPGERATLSCRASQSVSSSYLAWYQQKPGQAPRLLIYGASSRATGIPDRFSGSGSGTDFTLTISRLEPEDFAVYYCQQYGSSLWTFGQGTKVEIK

SEQ ID NO: 176 - protein, 108 aa, Artificial Sequence
  HIP1 Light Chain
EIVLTQSPGTLSLSPGERATLSCRASQSVSSSYLAWYQQKPGQAPRLLIYGASSRATGIPDRFSGSGSGTDFTLTISRLEPEDFAVYYCQQYGSSSWTFGQGTKVEIK

SEQ ID NO: 177 - protein, 109 aa, Artificial Sequence
  HIP1 Light Chain
EIVLTQSPGTLSLSPGERATLSCRASQSVSSSYLAWYQQKPGQAPRLLIYGASSRATGIPDRFSGSGSGTDFTLTISRLEPEDFAVYYCQQYGSSPTWTFGQGTKVEIK

SEQ ID NO: 178 - protein, 108 aa, Artificial Sequence; identical to SEQ ID NO: 173
  HIP2 Light Chain

SEQ ID NO: 179 - protein, 108 aa, Artificial Sequence; identical to SEQ ID NO: 175
  HIP2 Light Chain

SEQ ID NO: 180 - protein, 109 aa, Artificial Sequence; identical to SEQ ID NO: 174
  HIP2 Light Chain

SEQ ID NO: 181 - protein, 108 aa, Artificial Sequence; identical to SEQ ID NO: 176
  HIP2 Light Chain

SEQ ID NO: 182 - protein, 109 aa, Artificial Sequence; identical to SEQ ID NO: 177
  HIP2 Light Chain

SEQ ID NO: 183 - protein, 108 aa, Artificial Sequence; identical to SEQ ID NO: 173
  HIP3 Light Chain

SEQ ID NO: 184 - protein, 108 aa, Artificial Sequence; identical to SEQ ID NO: 175
  HIP3 Light Chain

SEQ ID NO: 185 - protein, 109 aa, Artificial Sequence; identical to SEQ ID NO: 174
  HIP3 Light Chain

SEQ ID NO: 186 - protein, 108 aa, Artificial Sequence; identical to SEQ ID NO: 176
  HIP3 Light Chain

SEQ ID NO: 187 - protein, 109 aa, Artificial Sequence; identical to SEQ ID NO: 177
  HIP3 Light Chain